European Patent Application EP 4 623 926 A1, published October 1, 2025. Title: Intranasal administration of BDNF for treatment of primary headaches. Applicant: Dompé farmaceutici SpA. Application EP. The sequence listing filed with the application follows.

SEQUENCE LISTING (12 sequences)

SEQ ID NO: 1 - DNA, 20 bp, synthetic construct
  source 1..20: mol_type = other DNA
aacctgccaagtatgatgac

SEQ ID NO: 2 - DNA, 19 bp, synthetic construct
  source 1..19: mol_type = other DNA
ggagttgctgttgaagtca

SEQ ID NO: 3 - DNA, 21 bp, synthetic construct
  source 1..21: mol_type = other DNA
cagtctcagctccaagtcatc

SEQ ID NO: 4 - DNA, 20 bp, synthetic construct
  source 1..20: mol_type = other DNA
ttccaaggttgacctcaaag

SEQ ID NO: 5 - DNA, 20 bp, synthetic construct
  source 1..20: mol_type = other DNA
caggcatgctgatggagttt

SEQ ID NO: 6 - DNA, 20 bp, synthetic construct
  source 1..20: mol_type = other DNA
tgctttctaaggcgggtgta

SEQ ID NO: 7 - DNA, 21 bp, synthetic construct
  source 1..21: mol_type = other DNA
caagacttctatgactgggac

SEQ ID NO: 8 - DNA, 20 bp, synthetic construct
  source 1..20: mol_type = other DNA
cttcgttaaggatttcgtgg

SEQ ID NO: 9 - DNA, 20 bp, synthetic construct
  source 1..20: mol_type = other DNA
cttccttgtgcaagtgtctg

SEQ ID NO: 10 - DNA, 21 bp, synthetic construct
  source 1..21: mol_type = other DNA
caggtcattctcctcactgtc

SEQ ID NO: 11 - DNA, 20 bp, synthetic construct
  source 1..20: mol_type = other DNA
gctcagcactgctatgttgc

SEQ ID NO: 12 - DNA, 20 bp, synthetic construct
  source 1..20: mol_type = other DNA
cagtagatgccgggtggttc